European Patent Application EP 4 488 365 A1, published January 8, 2025. Title: Production of hair follicle mesenchymal cells and use thereof. Applicant: National University Corporation YOKOHAMA Nationa l University. The sequence listing filed with the application follows.

SEQUENCE LISTING (4 sequences)

SEQ ID NO: 1 - DNA, 18 bp, synthetic construct
  misc_feature 1..18: note = ALP Forward Primer
  source 1..18: mol_type = other DNA
attgaccacgggcaccat

SEQ ID NO: 2 - DNA, 17 bp, synthetic construct
  misc_feature 1..17: note = ALP Reverse Primer
  source 1..17: mol_type = other DNA
ctccaccgcctcatgca

SEQ ID NO: 3 - DNA, 22 bp, synthetic construct
  misc_feature 1..22: note = GAPDH Forward Primer
  source 1..22: mol_type = other DNA
tggaaatcccatcaccatcttc

SEQ ID NO: 4 - DNA, 18 bp, synthetic construct
  misc_feature 1..18: note = GAPDH Reverse Primer
  source 1..18: mol_type = other DNA
cgccccacttgattttgg